European Patent Application EP 4 245 865 A1, published September 20, 2023. Title: BIOMARKERS FOR PREDICTING TREATMENT RESPONSE OF CANCER IMMUNOTHERAPY AND USES THEREOF. Applicant: Immune Oncia Therapeutics Inc. The sequence listing filed with the application follows.

SEQUENCE LISTING (10 sequences)

SEQ ID NO: 1 - protein, 121 aa, Artificial Sequence
  heavy chain (VH) variable domain of anti-PD-L1 antibody
QMQLVQSGAEVKKPGSSVKVSCKASGGTFSSYAYSWVRQAPGQGLEWMGGIIPSFGTANYAQKFQGRVTITADESTSTAYMELSSLRSEDTAVYYCARGPIVATITPLDYWGQGTLVTVSS

SEQ ID NO: 2 - protein, 108 aa, Artificial Sequence
  light chain (VL) variable domain of anti-PD-L1 antibody
SYVLTQPPSVSVAPGKTATIACGGENIGRKTVHWYQQKPGQAPVLVIYYDSDRPSGIPERFSGSNSGNTATLTISRVEAGDEADYYCLVWDSSSDHRIFGGGTKLTVL

SEQ ID NO: 3 - protein, 470 aa, Artificial Sequence
  heavy chain of anti-PD-L1 antibody
MEWSWVFLFFLSVTTGVHSQMQLVQSGAEVKKPGSSVKVSCKASGGTFSSYAYSWVRQAPGQGLEWMGGIIPSFGTANYAQKFQGRVTITADESTSTAYMELSSLRSEDTAVYYCARGPIVATITPLDYWGQGTLVTVSSASTKGPSVFPLAPSSKSTSGGTAALGCLVKDYFPEPVTVSWNSGALTSGVHTFPAVLQSSGLYSLSSVVTVPSSSLGTQTYICNVNHKPSNTKVDKRVEPKSCDKTHTCPPCPAPELLGGPSVFLFPPKPKDTLMISRTPEVTCVVVDVSHEDPEVKFNWYVDGVEVHNAKTKPREEQYNSTYRVVSVLTVLHQDWLNGKEYKCKVSNKALPAPIEKTISKAKGQPREPQVYTLPPSREEMTKNQVSLTCLVKGFYPSDIAVEWESNGQPENNYKTTPPVLDSDGSFFLYSKLTVDKSRWQQGNVFSCSVMHEALHNHYTQKSLSLSPGK

SEQ ID NO: 4 - protein, 234 aa, Artificial Sequence
  light chain of anti-PD-L1 antibody
MSVPTQVLGLLLLWLTDARCSYVLTQPPSVSVAPGKTATIACGGENIGRKTVHWYQQKPGQAPVLVIYYDSDRPSGIPERFSGSNSGNTATLTISRVEAGDEADYYCLVWDSSSDHRIFGGGTKLTVLGQPKAAPSVTLFPPSSEELQANKATLVCLISDFYPGAVTVAWKADSSPVKAGVETTTPSKQSNNKYAASSYLSLTPEQWKSHRSYSCQVTHEGSTVEKTVAPTECS

SEQ ID NO: 5 - protein, 5 aa, Artificial Sequence
  CDR1 (VH) of anti-PD-L1 antibody
SYAYS

SEQ ID NO: 6 - protein, 17 aa, Artificial Sequence
  CDR2 (VH) of anti-PD-L1 antibody
GIIPSFGTANYAQKFQG

SEQ ID NO: 7 - protein, 12 aa, Artificial Sequence
  CDR3 (VH) of anti-PD-L1 antibody
GPIVATITPLDY

SEQ ID NO: 8 - protein, 11 aa, Artificial Sequence
  CDR1 (VL) of anti-PD-L1 antibody
GGENIGRKTVH

SEQ ID NO: 9 - protein, 7 aa, Artificial Sequence
  CDR2 (VL) of anti-PD-L1 antibody
YDSDRPS

SEQ ID NO: 10 - protein, 11 aa, Artificial Sequence
  CDR3 (VL) of anti-PD-L1 antibody
LVWDSSSDHRI